European Patent Application EP 4 621 409 A1, published September 24, 2025. Title: NOVEL ANTIVIRAL PEPTIDE. Applicant: DAEHANNUPHARM CO., LTD. Application KR PCT/KR2023/018361, filed November 15, 2023. The sequence listing filed with the application follows.

SEQUENCE LISTING (304 sequences)

SEQ ID NO: 1 - protein, 18 aa, synthetic construct
  source 1..18: note = antiviral peptide candidate (or antiviral peptide)
ESLKNFWESLWKFFTHFF

SEQ ID NO: 2 - protein, 18 aa, synthetic construct
  source 1..18: note = antiviral peptide candidate (or antiviral peptide)
ITKFYKSFQDLWDMVIHI

SEQ ID NO: 3 - protein, 18 aa, synthetic construct
  source 1..18: note = antiviral peptide candidate (or antiviral peptide)
SFLDIVWSIIDIFKEFCK

SEQ ID NO: 4 - protein, 18 aa, synthetic construct
  source 1..18: note = antiviral peptide candidate (or antiviral peptide)
QSFLDIVWSIIDIFKEFC

SEQ ID NO: 5 - protein, 18 aa, synthetic construct
  source 1..18: note = antiviral peptide candidate (or antiviral peptide)
QDLCLRIFSSLVRILDLF

SEQ ID NO: 6 - protein, 18 aa, synthetic construct
  source 1..18: note = antiviral peptide candidate (or antiviral peptide)
LHGLIDGLEYWIRGYLDW

SEQ ID NO: 7 - protein, 18 aa, synthetic construct
  source 1..18: note = antiviral peptide candidate (or antiviral peptide)
LIDGLEYWIRGYLDWVVH

SEQ ID NO: 8 - protein, 18 aa, synthetic construct
  source 1..18: note = antiviral peptide candidate (or antiviral peptide)
NFIDKTFTVLADIILKIL

SEQ ID NO: 9 - protein, 18 aa, synthetic construct
  source 1..18: note = antiviral peptide candidate (or antiviral peptide)
NFIDKTFTIIADILLRII

SEQ ID NO: 10 - protein, 18 aa, synthetic construct
  source 1..18: note = antiviral peptide candidate (or antiviral peptide)
VFQWLWDWVKKIFNWLED

SEQ ID NO: 11 - protein, 18 aa, synthetic construct
  source 1..18: note = antiviral peptide candidate (or antiviral peptide)
LWDWVKKIFNWLEDLFLN

SEQ ID NO: 12 - protein, 18 aa, synthetic construct
  source 1..18: note = antiviral peptide candidate (or antiviral peptide)
WVKKIFNWLEDLFLNFTG

SEQ ID NO: 13 - protein, 18 aa, synthetic construct
  source 1..18: note = antiviral peptide candidate (or antiviral peptide)
VVIYGIIGFLDDFLKIFK

SEQ ID NO: 14 - protein, 18 aa, synthetic construct
  source 1..18: note = antiviral peptide candidate (or antiviral peptide)
FFLRWLYSVSDYLSDFWE

SEQ ID NO: 15 - protein, 18 aa, synthetic construct
  source 1..18: note = antiviral peptide candidate (or antiviral peptide)
RWLYSVSDYLSDFWESLL

SEQ ID NO: 16 - protein, 18 aa, synthetic construct
  source 1..18: note = antiviral peptide candidate (or antiviral peptide)
DALWRLWLGFFREHFAAI

SEQ ID NO: 17 - protein, 18 aa, synthetic construct
  source 1..18: note = antiviral peptide candidate (or antiviral peptide)
SEWTGILDRLLKWVGLLV

SEQ ID NO: 18 - protein, 18 aa, synthetic construct
  source 1..18: note = antiviral peptide candidate (or antiviral peptide)
TGILDRLLKWVGLLVDIV

SEQ ID NO: 19 - protein, 18 aa, synthetic construct
  source 1..18: note = antiviral peptide candidate (or antiviral peptide)
VELIDDLYRKLYSWFLHI

SEQ ID NO: 20 - protein, 18 aa, synthetic construct
  source 1..18: note = antiviral peptide candidate (or antiviral peptide)
IDDLYRKLYSWFLHILTF

SEQ ID NO: 21 - protein, 18 aa, synthetic construct
  source 1..18: note = antiviral peptide candidate (or antiviral peptide)
MGIFQAFADVFKLLFKEI

SEQ ID NO: 22 - protein, 18 aa, synthetic construct
  source 1..18: note = antiviral peptide candidate (or antiviral peptide)
AHFGFFWRWFDEIFTLLD

SEQ ID NO: 23 - protein, 18 aa, synthetic construct
  source 1..18: note = antiviral peptide candidate (or antiviral peptide)
WEALKYWWNLLQYWSKEL

SEQ ID NO: 24 - protein, 18 aa, synthetic construct
  source 1..18: note = antiviral peptide candidate (or antiviral peptide)
FQFIQKLIDDLLHVIEGL

SEQ ID NO: 25 - protein, 18 aa, synthetic construct
  source 1..18: note = antiviral peptide candidate (or antiviral peptide)
IQKLIDDLLHVIEGLVLI

SEQ ID NO: 26 - protein, 18 aa, synthetic construct
  source 1..18: note = antiviral peptide candidate (or antiviral peptide)
FDFIEKFSHVLFDIVGII

SEQ ID NO: 27 - protein, 18 aa, synthetic construct
  source 1..18: note = antiviral peptide candidate (or antiviral peptide)
IEKFSHVLFDIVGIIMKV

SEQ ID NO: 28 - protein, 18 aa, synthetic construct
  source 1..18: note = antiviral peptide candidate (or antiviral peptide)
FDFIKSIIIGIVEGLTEF

SEQ ID NO: 29 - protein, 18 aa, synthetic construct
  source 1..18: note = antiviral peptide candidate (or antiviral peptide)
IDILIRFYHLFESIYKYI

SEQ ID NO: 30 - protein, 18 aa, synthetic construct
  source 1..18: note = antiviral peptide candidate (or antiviral peptide)
LIRFYHLFESIYKYIMDL

SEQ ID NO: 31 - protein, 18 aa, synthetic construct
  source 1..18: note = antiviral peptide candidate (or antiviral peptide)
QIGKDISNLLFDIWRVWL

SEQ ID NO: 32 - protein, 18 aa, synthetic construct
  source 1..18: note = antiviral peptide candidate (or antiviral peptide)
ISNLLFDIWRVWLEKLGE

SEQ ID NO: 33 - protein, 18 aa, synthetic construct
  source 1..18: note = antiviral peptide candidate (or antiviral peptide)
LLSMFLVMIQWWRDIVRE

SEQ ID NO: 34 - protein, 18 aa, synthetic construct
  source 1..18: note = antiviral peptide candidate (or antiviral peptide)
ILDTSVQFWYEFIDYIMR

SEQ ID NO: 35 - protein, 18 aa, synthetic construct
  source 1..18: note = antiviral peptide candidate (or antiviral peptide)
TSVQFWYEFIDYIMRVIE

SEQ ID NO: 36 - protein, 18 aa, synthetic construct
  source 1..18: note = antiviral peptide candidate (or antiviral peptide)
EILGAFFHKFEKFFDLFM

SEQ ID NO: 37 - protein, 18 aa, synthetic construct
  source 1..18: note = antiviral peptide candidate (or antiviral peptide)
FGLVKLWVEKIVSFIEQF

SEQ ID NO: 38 - protein, 18 aa, synthetic construct
  source 1..18: note = antiviral peptide candidate (or antiviral peptide)
VKLWVEKIVSFIEQFLNF

SEQ ID NO: 39 - protein, 18 aa, synthetic construct
  source 1..18: note = antiviral peptide candidate (or antiviral peptide)
LFYLLSRLWFGLLETFRD

SEQ ID NO: 40 - protein, 18 aa, synthetic construct
  source 1..18: note = antiviral peptide candidate (or antiviral peptide)
LLSRLWFGLLETFRDILV

SEQ ID NO: 41 - protein, 18 aa, synthetic construct
  source 1..18: note = antiviral peptide candidate (or antiviral peptide)
RFVQGVDMFLETLWKVWM

SEQ ID NO: 42 - protein, 18 aa, synthetic construct
  source 1..18: note = antiviral peptide candidate (or antiviral peptide)
QGVDMFLETLWKVWMELL

SEQ ID NO: 43 - protein, 18 aa, synthetic construct
  source 1..18: note = antiviral peptide candidate (or antiviral peptide)
WSEIFRELFSLLGRIWSS

SEQ ID NO: 44 - protein, 18 aa, synthetic construct
  source 1..18: note = antiviral peptide candidate (or antiviral peptide)
LALEKYWIEWLEKWQMLL

SEQ ID NO: 45 - protein, 18 aa, synthetic construct
  source 1..18: note = antiviral peptide candidate (or antiviral peptide)
FFHLWLNILAELLRFGDR

SEQ ID NO: 46 - protein, 18 aa, synthetic construct
  source 1..18: note = antiviral peptide candidate (or antiviral peptide)
ILDFFVGFIDWLVRYLNK

SEQ ID NO: 47 - protein, 18 aa, synthetic construct
  source 1..18: note = antiviral peptide candidate (or antiviral peptide)
MDFIRAIILGIIEGITEW

SEQ ID NO: 48 - protein, 18 aa, synthetic construct
  source 1..18: note = antiviral peptide candidate (or antiviral peptide)
DHWHNLFIKLFKYYYDII

SEQ ID NO: 49 - protein, 18 aa, synthetic construct
  source 1..18: note = antiviral peptide candidate (or antiviral peptide)
YNLFDLLIYIWNKIFDDY

SEQ ID NO: 50 - protein, 18 aa, synthetic construct
  source 1..18: note = antiviral peptide candidate (or antiviral peptide)
DIFQDLLKEVIFVLSKIL

SEQ ID NO: 51 - protein, 18 aa, synthetic construct
  source 1..18: note = antiviral peptide candidate (or antiviral peptide)
LEILVQILRYWIKDVSFF

SEQ ID NO: 52 - protein, 18 aa, synthetic construct
  source 1..18: note = antiviral peptide candidate (or antiviral peptide)
LHIISYMGDIFKLIKEFW

SEQ ID NO: 53 - protein, 18 aa, synthetic construct
  source 1..18: note = antiviral peptide candidate (or antiviral peptide)
EVWIEGLRSYLLDWWNFL

SEQ ID NO: 54 - protein, 18 aa, synthetic construct
  source 1..18: note = antiviral peptide candidate (or antiviral peptide)
LNFIGVLVDSLKEILNEW

SEQ ID NO: 55 - protein, 18 aa, synthetic construct
  source 1..18: note = antiviral peptide candidate (or antiviral peptide)
GGFWDSIKALWRNLIDFL

SEQ ID NO: 56 - protein, 18 aa, synthetic construct
  source 1..18: note = antiviral peptide candidate (or antiviral peptide)
NFIYKELEQIIDLFMVLI

SEQ ID NO: 57 - protein, 18 aa, synthetic construct
  source 1..18: note = antiviral peptide candidate (or antiviral peptide)
FFDSIRILWTKIINGLVD

SEQ ID NO: 58 - protein, 18 aa, synthetic construct
  source 1..18: note = antiviral peptide candidate (or antiviral peptide)
MLMEQFLDYIGKLLFKIF

SEQ ID NO: 59 - protein, 18 aa, synthetic construct
  source 1..18: note = antiviral peptide candidate (or antiviral peptide)
EQFLDYIGKLLFKIFMTI

SEQ ID NO: 60 - protein, 18 aa, synthetic construct
  source 1..18: note = antiviral peptide candidate (or antiviral peptide)
KSLNFVLAAWIRILEEIL

SEQ ID NO: 61 - protein, 18 aa, synthetic construct
  source 1..18: note = antiviral peptide candidate (or antiviral peptide)
ETFKEFVHVWFKSIFNWI

SEQ ID NO: 62 - protein, 18 aa, synthetic construct
  source 1..18: note = antiviral peptide candidate (or antiviral peptide)
FDFFKIVGEIFGLFENYF

SEQ ID NO: 63 - protein, 18 aa, synthetic construct
  source 1..18: note = antiviral peptide candidate (or antiviral peptide)
TIVSRVLGKVLDFWVDFI

SEQ ID NO: 64 - protein, 18 aa, synthetic construct
  source 1..18: note = antiviral peptide candidate (or antiviral peptide)
TTLMKFVELWFKDVFNWM

SEQ ID NO: 65 - protein, 18 aa, synthetic construct
  source 1..18: note = antiviral peptide candidate (or antiviral peptide)
QWFDLLKDIFSKFTIFLQ

SEQ ID NO: 66 - protein, 18 aa, synthetic construct
  source 1..18: note = antiviral peptide candidate (or antiviral peptide)
LLKELLDLLQDMVVMLLS

SEQ ID NO: 67 - protein, 18 aa, synthetic construct
  source 1..18: note = antiviral peptide candidate (or antiviral peptide)
AIFTFLHKLVEVLSDYLK

SEQ ID NO: 68 - protein, 18 aa, synthetic construct
  source 1..18: note = antiviral peptide candidate (or antiviral peptide)
AIMKKIIDFYGQWVDSFI

SEQ ID NO: 69 - protein, 18 aa, synthetic construct
  source 1..18: note = antiviral peptide candidate (or antiviral peptide)
ANINDILMKIIKIFDAIL

SEQ ID NO: 70 - protein, 18 aa, synthetic construct
  source 1..18: note = antiviral peptide candidate (or antiviral peptide)
AVTWDILLDIIERLLQQL

SEQ ID NO: 71 - protein, 18 aa, synthetic construct
  source 1..18: note = antiviral peptide candidate (or antiviral peptide)
WDILLDIIERLLQQLQNL

SEQ ID NO: 72 - protein, 18 aa, synthetic construct
  source 1..18: note = antiviral peptide candidate (or antiviral peptide)
LVLYGLIGFLDDFLKVFR

SEQ ID NO: 73 - protein, 18 aa, synthetic construct
  source 1..18: note = antiviral peptide candidate (or antiviral peptide)
IDFFDKVSHVFFKIIGYI

SEQ ID NO: 74 - protein, 18 aa, synthetic construct
  source 1..18: note = antiviral peptide candidate (or antiviral peptide)
IIELIKGIILGIVEGLTE

SEQ ID NO: 75 - protein, 18 aa, synthetic construct
  source 1..18: note = antiviral peptide candidate (or antiviral peptide)
HEVLDFLDNLMISIFKIL

SEQ ID NO: 76 - protein, 18 aa, synthetic construct
  source 1..18: note = antiviral peptide candidate (or antiviral peptide)
SIWQLVLEQFDDLLVKIL

SEQ ID NO: 77 - protein, 18 aa, synthetic construct
  source 1..18: note = antiviral peptide candidate (or antiviral peptide)
DIIDRFVDWITMTFGGFF

SEQ ID NO: 78 - protein, 18 aa, synthetic construct
  source 1..18: note = antiviral peptide candidate (or antiviral peptide)
YEVYRVFSDILHIFLKLI

SEQ ID NO: 79 - protein, 18 aa, synthetic construct
  source 1..18: note = antiviral peptide candidate (or antiviral peptide)
VVGLIIKWFDWIYELGKQ

SEQ ID NO: 80 - protein, 18 aa, synthetic construct
  source 1..18: note = antiviral peptide candidate (or antiviral peptide)
DMLGSLYKILENILIIFR

SEQ ID NO: 81 - protein, 18 aa, synthetic construct
  source 1..18: note = antiviral peptide candidate (or antiviral peptide)
KKLVEYILDIFLKLSEIL

SEQ ID NO: 82 - protein, 18 aa, synthetic construct
  source 1..18: note = antiviral peptide candidate (or antiviral peptide)
MTVISLFKNLIEIFEKYL

SEQ ID NO: 83 - protein, 18 aa, synthetic construct
  source 1..18: note = antiviral peptide candidate (or antiviral peptide)
VDLFSDFVTLFRKLMMIL

SEQ ID NO: 84 - protein, 18 aa, synthetic construct
  source 1..18: note = antiviral peptide candidate (or antiviral peptide)
QDLKEIISYIFDIIKIII

SEQ ID NO: 85 - protein, 18 aa, synthetic construct
  source 1..18: note = antiviral peptide candidate (or antiviral peptide)
DLLIDILKYLVRLTEDII

SEQ ID NO: 86 - protein, 18 aa, synthetic construct
  source 1..18: note = antiviral peptide candidate (or antiviral peptide)
DSIIDLFKDFMLTFRQFF

SEQ ID NO: 87 - protein, 18 aa, synthetic construct
  source 1..18: note = antiviral peptide candidate (or antiviral peptide)
FWKDIINLIKGFILSIID

SEQ ID NO: 88 - protein, 18 aa, synthetic construct
  source 1..18: note = antiviral peptide candidate (or antiviral peptide)
MEFFQEYYDIIRLWSTIL

SEQ ID NO: 89 - protein, 18 aa, synthetic construct
  source 1..18: note = antiviral peptide candidate (or antiviral peptide)
DVLVKAWAMWGDYLENIF

SEQ ID NO: 90 - protein, 18 aa, synthetic construct
  source 1..18: note = antiviral peptide candidate (or antiviral peptide)
KFLKAVFELWEFIKDFLV

SEQ ID NO: 91 - protein, 18 aa, synthetic construct
  source 1..18: note = antiviral peptide candidate (or antiviral peptide)
LKEWLDYYNWLSRLIEFF

SEQ ID NO: 92 - protein, 18 aa, synthetic construct
  source 1..18: note = antiviral peptide candidate (or antiviral peptide)
TEFIKMFKSFVDLLFEVV

SEQ ID NO: 93 - protein, 18 aa, synthetic construct
  source 1..18: note = antiviral peptide candidate (or antiviral peptide)
VLILKTIRELTSFFIDLL

SEQ ID NO: 94 - protein, 18 aa, synthetic construct
  source 1..18: note = antiviral peptide candidate (or antiviral peptide)
EILDFFMTLFGSILTDIR

SEQ ID NO: 95 - protein, 18 aa, synthetic construct
  source 1..18: note = antiviral peptide candidate (or antiviral peptide)
FTTILSDFQSFLERLLDI

SEQ ID NO: 96 - protein, 18 aa, synthetic construct
  source 1..18: note = antiviral peptide candidate (or antiviral peptide)
TEILKQFLTHFDTIFEVF

SEQ ID NO: 97 - protein, 18 aa, synthetic construct
  source 1..18: note = antiviral peptide candidate (or antiviral peptide)
ELIDELYQKVYRWFMQIF

SEQ ID NO: 98 - protein, 18 aa, synthetic construct
  source 1..18: note = antiviral peptide candidate (or antiviral peptide)
LEQLMYLIEEFVKYLIRF

SEQ ID NO: 99 - protein, 18 aa, synthetic construct
  source 1..18: note = antiviral peptide candidate (or antiviral peptide)
SELMRWIISEIYAVWKIF

SEQ ID NO: 100 - protein, 18 aa, synthetic construct
  source 1..18: note = antiviral peptide candidate (or antiviral peptide)
IKFLKEFIEFLREYINVI

SEQ ID NO: 101 - protein, 18 aa, synthetic construct
  source 1..18: note = antiviral peptide candidate (or antiviral peptide)
SWKEIVNLLYELLASLIR

SEQ ID NO: 102 - protein, 18 aa, synthetic construct
  source 1..18: note = antiviral peptide candidate (or antiviral peptide)
YITAILVLWSRMMKEILD

SEQ ID NO: 103 - protein, 18 aa, synthetic construct
  source 1..18: note = antiviral peptide candidate (or antiviral peptide)
IAFGIIGFLDDILKIIHR

SEQ ID NO: 104 - protein, 18 aa, synthetic construct
  source 1..18: note = antiviral peptide candidate (or antiviral peptide)
FWRRHVFIWISFIDSYFE

SEQ ID NO: 105 - protein, 18 aa, synthetic construct
  source 1..18: note = antiviral peptide candidate (or antiviral peptide)
GKIFKVLYDSFMLLWNEW

SEQ ID NO: 106 - protein, 18 aa, synthetic construct
  source 1..18: note = antiviral peptide candidate (or antiviral peptide)
GWFGFISDAMELVLKILK

SEQ ID NO: 107 - protein, 18 aa, synthetic construct
  source 1..18: note = antiviral peptide candidate (or antiviral peptide)
KVIFDVIESFSKVIFGVI

SEQ ID NO: 108 - protein, 18 aa, synthetic construct
  source 1..18: note = antiviral peptide candidate (or antiviral peptide)
VILDLFKEIIDEVLKGII

SEQ ID NO: 109 - protein, 18 aa, synthetic construct
  source 1..18: note = antiviral peptide candidate (or antiviral peptide)
FLDALLKILEGWLYTYAK

SEQ ID NO: 110 - protein, 18 aa, synthetic construct
  source 1..18: note = antiviral peptide candidate (or antiviral peptide)
WSEILREFLNLISLIWSR

SEQ ID NO: 111 - protein, 18 aa, synthetic construct
  source 1..18: note = antiviral peptide candidate (or antiviral peptide)
IFLYLVDQIYDIIRMIEK

SEQ ID NO: 112 - protein, 18 aa, synthetic construct
  source 1..18: note = antiviral peptide candidate (or antiviral peptide)
YIYLILKFIQDIYNDIYR

SEQ ID NO: 113 - protein, 18 aa, synthetic construct
  source 1..18: note = antiviral peptide candidate (or antiviral peptide)
FQFIEKFSEIMFELVRMI

SEQ ID NO: 114 - protein, 18 aa, synthetic construct
  source 1..18: note = antiviral peptide candidate (or antiviral peptide)
FSFWVWLDNIIDLVKKYI

SEQ ID NO: 115 - protein, 18 aa, synthetic construct
  source 1..18: note = antiviral peptide candidate (or antiviral peptide)
YTSFVDVFFKIVDYLNKW

SEQ ID NO: 116 - protein, 18 aa, synthetic construct
  source 1..18: note = antiviral peptide candidate (or antiviral peptide)
FTFWTWLEAILDLIKKHI

SEQ ID NO: 117 - protein, 18 aa, synthetic construct
  source 1..18: note = antiviral peptide candidate (or antiviral peptide)
MFVETLWKVWTELLDVLG

SEQ ID NO: 118 - protein, 18 aa, synthetic construct
  source 1..18: note = antiviral peptide candidate (or antiviral peptide)
VLVGMIIKWFDWLYEMGK

SEQ ID NO: 119 - protein, 18 aa, synthetic construct
  source 1..18: note = antiviral peptide candidate (or antiviral peptide)
GILINVINDFERQWLRIF

SEQ ID NO: 120 - protein, 18 aa, synthetic construct
  source 1..18: note = antiviral peptide candidate (or antiviral peptide)
GLQNFLEWVVDFIRGIIK

SEQ ID NO: 121 - protein, 18 aa, synthetic construct
  source 1..18: note = antiviral peptide candidate (or antiviral peptide)
TRIVDWYDLVYGLLDGWW

SEQ ID NO: 122 - protein, 18 aa, synthetic construct
  source 1..18: note = antiviral peptide candidate (or antiviral peptide)
GLLEIIVILWKNIHRSLE

SEQ ID NO: 123 - protein, 18 aa, synthetic construct
  source 1..18: note = antiviral peptide candidate (or antiviral peptide)
LIWELIKQILKGISYIHD

SEQ ID NO: 124 - protein, 18 aa, synthetic construct
  source 1..18: note = antiviral peptide candidate (or antiviral peptide)
YLWLDLRGFWTQIFEEIV

SEQ ID NO: 125 - protein, 18 aa, synthetic construct
  source 1..18: note = antiviral peptide candidate (or antiviral peptide)
LLKIVSALWEKWLSLLEA

SEQ ID NO: 126 - protein, 18 aa, synthetic construct
  source 1..18: note = antiviral peptide candidate (or antiviral peptide)
HWWFEGVKWLGRVLELLY

SEQ ID NO: 127 - protein, 18 aa, synthetic construct
  source 1..18: note = antiviral peptide candidate (or antiviral peptide)
FSELLRLTRTLLGIIDCI

SEQ ID NO: 128 - protein, 18 aa, synthetic construct
  source 1..18: note = antiviral peptide candidate (or antiviral peptide)
QIIDWYSGLVRRWVIWYE

SEQ ID NO: 129 - protein, 18 aa, synthetic construct
  source 1..18: note = antiviral peptide candidate (or antiviral peptide)
ECAEKILETWGELLSKWH

SEQ ID NO: 130 - protein, 18 aa, synthetic construct
  source 1..18: note = antiviral peptide candidate (or antiviral peptide)
IRTLFDEITRILNHLLWL

SEQ ID NO: 131 - protein, 18 aa, synthetic construct
  source 1..18: note = antiviral peptide candidate (or antiviral peptide)
TLYAFFLTLIREIVKGIE

SEQ ID NO: 132 - protein, 18 aa, synthetic construct
  source 1..18: note = antiviral peptide candidate (or antiviral peptide)
WKEWWKVFYTIVDYINQI

SEQ ID NO: 133 - protein, 18 aa, synthetic construct
  source 1..18: note = antiviral peptide candidate (or antiviral peptide)
WKKWWQVFYTVVDYVDQI

SEQ ID NO: 134 - protein, 18 aa, synthetic construct
  source 1..18: note = antiviral peptide candidate (or antiviral peptide)
VKLGSIYFSFFDDFFRII

SEQ ID NO: 135 - protein, 18 aa, synthetic construct
  source 1..18: note = antiviral peptide candidate (or antiviral peptide)
KLMVDFFNILNEIVMKLV

SEQ ID NO: 136 - protein, 18 aa, synthetic construct
  source 1..18: note = antiviral peptide candidate (or antiviral peptide)
YKWFAFFKDVTDFISHLF

SEQ ID NO: 137 - protein, 18 aa, synthetic construct
  source 1..18: note = antiviral peptide candidate (or antiviral peptide)
LDAIGDLLLDFLLLLNKW

SEQ ID NO: 138 - protein, 18 aa, synthetic construct
  source 1..18: note = antiviral peptide candidate (or antiviral peptide)
LTLLLLTMVQWWRDIIRE

SEQ ID NO: 139 - protein, 18 aa, synthetic construct
  source 1..18: note = antiviral peptide candidate (or antiviral peptide)
TLLRAVETLFSLWLEFMR

SEQ ID NO: 140 - protein, 18 aa, synthetic construct
  source 1..18: note = antiviral peptide candidate (or antiviral peptide)
LRLWEIIARYVEGIVHLF

SEQ ID NO: 141 - protein, 18 aa, synthetic construct
  source 1..18: note = antiviral peptide candidate (or antiviral peptide)
WLDNIIDLVKKYILALWN

SEQ ID NO: 142 - protein, 18 aa, synthetic construct
  source 1..18: note = antiviral peptide candidate (or antiviral peptide)
WFEALLGYISAVIEYFEK

SEQ ID NO: 143 - protein, 18 aa, synthetic construct
  source 1..18: note = antiviral peptide candidate (or antiviral peptide)
DFWSKLVYFFAEIIRFLS

SEQ ID NO: 144 - protein, 18 aa, synthetic construct
  source 1..18: note = antiviral peptide candidate (or antiviral peptide)
AKNIIKLLLELIEVILNV

SEQ ID NO: 145 - protein, 18 aa, synthetic construct
  source 1..18: note = antiviral peptide candidate (or antiviral peptide)
LEEILEVIISLFKKLNLI

SEQ ID NO: 146 - protein, 18 aa, synthetic construct
  source 1..18: note = antiviral peptide candidate (or antiviral peptide)
LLVKILKLIINELSNVME

SEQ ID NO: 147 - protein, 18 aa, synthetic construct
  source 1..18: note = antiviral peptide candidate (or antiviral peptide)
ALLIYFRRDWVDLIGGWL

SEQ ID NO: 148 - protein, 18 aa, synthetic construct
  source 1..18: note = antiviral peptide candidate (or antiviral peptide)
IQWFEVLDGLLGRYWKAL

SEQ ID NO: 149 - protein, 18 aa, synthetic construct
  source 1..18: note = antiviral peptide candidate (or antiviral peptide)
ATWQDWFHRWLEILDSSL

SEQ ID NO: 150 - protein, 18 aa, synthetic construct
  source 1..18: note = antiviral peptide candidate (or antiviral peptide)
LWKSLDSWASLILQWFED

SEQ ID NO: 151 - protein, 18 aa, synthetic construct
  source 1..18: note = antiviral peptide candidate (or antiviral peptide)
DVTRLLELILDVLAYIIS

SEQ ID NO: 152 - protein, 18 aa, synthetic construct
  source 1..18: note = antiviral peptide candidate (or antiviral peptide)
DEFLDFAALLFGWFRKFV

SEQ ID NO: 153 - protein, 18 aa, synthetic construct
  source 1..18: note = antiviral peptide candidate (or antiviral peptide)
DEILGRLLKILFVLFVDL

SEQ ID NO: 154 - protein, 18 aa, synthetic construct
  source 1..18: note = antiviral peptide candidate (or antiviral peptide)
FRMFIGDLEKIVNLLLSL

SEQ ID NO: 155 - protein, 18 aa, synthetic construct
  source 1..18: note = antiviral peptide candidate (or antiviral peptide)
ILLKFLESVGGVLLDILR

SEQ ID NO: 156 - protein, 18 aa, synthetic construct
  source 1..18: note = antiviral peptide candidate (or antiviral peptide)
LIVILDDSFLELLRLFIK

SEQ ID NO: 157 - protein, 18 aa, synthetic construct
  source 1..18: note = antiviral peptide candidate (or antiviral peptide)
LLFGLLGFLDDYLKVVLR

SEQ ID NO: 158 - protein, 18 aa, synthetic construct
  source 1..18: note = antiviral peptide candidate (or antiviral peptide)
LFYGFIGFLDDFVSIVKK

SEQ ID NO: 159 - protein, 18 aa, synthetic construct
  source 1..18: note = antiviral peptide candidate (or antiviral peptide)
IEIMDFVIGVLDSIAKIF

SEQ ID NO: 160 - protein, 18 aa, synthetic construct
  source 1..18: note = antiviral peptide candidate (or antiviral peptide)
IEQLVEYTKIILDFIISW

SEQ ID NO: 161 - protein, 18 aa, synthetic construct
  source 1..18: note = antiviral peptide candidate (or antiviral peptide)
KIFIGLLELIEDIFHGTF

SEQ ID NO: 162 - protein, 18 aa, synthetic construct
  source 1..18: note = antiviral peptide candidate (or antiviral peptide)
FRYLIEAINSFVKVFELW

SEQ ID NO: 163 - protein, 18 aa, synthetic construct
  source 1..18: note = antiviral peptide candidate (or antiviral peptide)
INLLLKIVFELSKLIDDF

SEQ ID NO: 164 - protein, 18 aa, synthetic construct
  source 1..18: note = antiviral peptide candidate (or antiviral peptide)
NFIDRVFTVISDLILKLL

SEQ ID NO: 165 - protein, 18 aa, synthetic construct
  source 1..18: note = antiviral peptide candidate (or antiviral peptide)
SIFELILNQFDDLLVKIL

SEQ ID NO: 166 - protein, 18 aa, synthetic construct
  source 1..18: note = antiviral peptide candidate (or antiviral peptide)
DIIKDFAKFFTIFFGITF

SEQ ID NO: 167 - protein, 18 aa, synthetic construct
  source 1..18: note = antiviral peptide candidate (or antiviral peptide)
WRGMLIKILSFIEGYIDF

SEQ ID NO: 168 - protein, 18 aa, synthetic construct
  source 1..18: note = antiviral peptide candidate (or antiviral peptide)
LKDWLGFWLSLYQRFIEN

SEQ ID NO: 169 - protein, 18 aa, synthetic construct
  source 1..18: note = antiviral peptide candidate (or antiviral peptide)
NDILKVLSEWLTDLFTII

SEQ ID NO: 170 - protein, 18 aa, synthetic construct
  source 1..18: note = antiviral peptide candidate (or antiviral peptide)
DIWVNVLVSFITLLREWR

SEQ ID NO: 171 - protein, 18 aa, synthetic construct
  source 1..18: note = antiviral peptide candidate (or antiviral peptide)
DKIVLFILSILEKIYNLL

SEQ ID NO: 172 - protein, 18 aa, synthetic construct
  source 1..18: note = antiviral peptide candidate (or antiviral peptide)
EDILFSILYLLKKIANLI

SEQ ID NO: 173 - protein, 18 aa, synthetic construct
  source 1..18: note = antiviral peptide candidate (or antiviral peptide)
ILADILVKLLDEIKYILK

SEQ ID NO: 174 - protein, 18 aa, synthetic construct
  source 1..18: note = antiviral peptide candidate (or antiviral peptide)
LLEYIDLVYNILISILKK

SEQ ID NO: 175 - protein, 18 aa, synthetic construct
  source 1..18: note = antiviral peptide candidate (or antiviral peptide)
MLESLINKLITLIDFIVD

SEQ ID NO: 176 - protein, 18 aa, synthetic construct
  source 1..18: note = antiviral peptide candidate (or antiviral peptide)
DLIHIILDKIIDTLVHFM

SEQ ID NO: 177 - protein, 18 aa, synthetic construct
  source 1..18: note = antiviral peptide candidate (or antiviral peptide)
LRLLSNYFESMIDIFVKL

SEQ ID NO: 178 - protein, 18 aa, synthetic construct
  source 1..18: note = antiviral peptide candidate (or antiviral peptide)
DVLLRVFVEGWTHLVRLL

SEQ ID NO: 179 - protein, 18 aa, synthetic construct
  source 1..18: note = antiviral peptide candidate (or antiviral peptide)
DVMADQFVTFLEKWFKLF

SEQ ID NO: 180 - protein, 18 aa, synthetic construct
  source 1..18: note = antiviral peptide candidate (or antiviral peptide)
DWQALWEELKSIFVFWIN

SEQ ID NO: 181 - protein, 18 aa, synthetic construct
  source 1..18: note = antiviral peptide candidate (or antiviral peptide)
ESIWEFIKSLLDAWSGWV

SEQ ID NO: 182 - protein, 18 aa, synthetic construct
  source 1..18: note = antiviral peptide candidate (or antiviral peptide)
FWEIFVVWLKQFIDIENS

SEQ ID NO: 183 - protein, 18 aa, synthetic construct
  source 1..18: note = antiviral peptide candidate (or antiviral peptide)
WFIKKLNTWLDVILDEWK

SEQ ID NO: 184 - protein, 18 aa, synthetic construct
  source 1..18: note = antiviral peptide candidate (or antiviral peptide)
EALMLIYKLFWDEFSSWL

SEQ ID NO: 185 - protein, 18 aa, synthetic construct
  source 1..18: note = antiviral peptide candidate (or antiviral peptide)
WDCVQDIWEYIFRTAMKI

SEQ ID NO: 186 - protein, 18 aa, synthetic construct
  source 1..18: note = antiviral peptide candidate (or antiviral peptide)
EEIAVILRIMEKLWHVFM

SEQ ID NO: 187 - protein, 18 aa, synthetic construct
  source 1..18: note = antiviral peptide candidate (or antiviral peptide)
EDVSEVLAHIGTCLRKIF

SEQ ID NO: 188 - protein, 18 aa, synthetic construct
  source 1..18: note = antiviral peptide candidate (or antiviral peptide)
EFWNRWHMSLSFWFRDFV

SEQ ID NO: 189 - protein, 18 aa, synthetic construct
  source 1..18: note = antiviral peptide candidate (or antiviral peptide)
EGILSFILISLKDFLRVF

SEQ ID NO: 190 - protein, 18 aa, synthetic construct
  source 1..18: note = antiviral peptide candidate (or antiviral peptide)
IVHLLNELFTKFDRLIGI

SEQ ID NO: 191 - protein, 18 aa, synthetic construct
  source 1..18: note = antiviral peptide candidate (or antiviral peptide)
FTNFHRQLFCWIDKWIDL

SEQ ID NO: 192 - protein, 18 aa, synthetic construct
  source 1..18: note = antiviral peptide candidate (or antiviral peptide)
LWEAIETFIGEIIAIFYK

SEQ ID NO: 193 - protein, 18 aa, synthetic construct
  source 1..18: note = antiviral peptide candidate (or antiviral peptide)
WEKTLSLIGEVIEIWMLV

SEQ ID NO: 194 - protein, 18 aa, synthetic construct
  source 1..18: note = antiviral peptide candidate (or antiviral peptide)
EILREFMTLISHIWSQIK

SEQ ID NO: 195 - protein, 18 aa, synthetic construct
  source 1..18: note = antiviral peptide candidate (or antiviral peptide)
QDILSKLYLLLARVFEIW

SEQ ID NO: 196 - protein, 18 aa, synthetic construct
  source 1..18: note = antiviral peptide candidate (or antiviral peptide)
SFIRKGIEAWFTLLMELI

SEQ ID NO: 197 - protein, 18 aa, synthetic construct
  source 1..18: note = antiviral peptide candidate (or antiviral peptide)
EMFALIFEYIDRIFSIVR

SEQ ID NO: 198 - protein, 18 aa, synthetic construct
  source 1..18: note = antiviral peptide candidate (or antiviral peptide)
ENWKDFFLIFWQKYFNVW

SEQ ID NO: 199 - protein, 18 aa, synthetic construct
  source 1..18: note = antiviral peptide candidate (or antiviral peptide)
LNKYFFEWFQAIKGFVEW

SEQ ID NO: 200 - protein, 18 aa, synthetic construct
  source 1..18: note = antiviral peptide candidate (or antiviral peptide)
FGLLQSFADFLKYIVKEI

SEQ ID NO: 201 - protein, 18 aa, synthetic construct
  source 1..18: note = antiviral peptide candidate (or antiviral peptide)
KIMFTFVKELLNYLDGFI

SEQ ID NO: 202 - protein, 18 aa, synthetic construct
  source 1..18: note = antiviral peptide candidate (or antiviral peptide)
ETLVRLFRFFLGEWYAVL

SEQ ID NO: 203 - protein, 18 aa, synthetic construct
  source 1..18: note = antiviral peptide candidate (or antiviral peptide)
EVILASWYRIYTKIMDLI

SEQ ID NO: 204 - protein, 18 aa, synthetic construct
  source 1..18: note = antiviral peptide candidate (or antiviral peptide)
IVLEIIHHFVEILDRYFG

SEQ ID NO: 205 - protein, 18 aa, synthetic construct
  source 1..18: note = antiviral peptide candidate (or antiviral peptide)
KIVIGLLEFVEDIFHGLY

SEQ ID NO: 206 - protein, 18 aa, synthetic construct
  source 1..18: note = antiviral peptide candidate (or antiviral peptide)
EYIDNIIEYIINILKLTI

SEQ ID NO: 207 - protein, 18 aa, synthetic construct
  source 1..18: note = antiviral peptide candidate (or antiviral peptide)
IIIITDLLENLKELIIKI

SEQ ID NO: 208 - protein, 18 aa, synthetic construct
  source 1..18: note = antiviral peptide candidate (or antiviral peptide)
FAKDIWRILTAWFAGLAD

SEQ ID NO: 209 - protein, 18 aa, synthetic construct
  source 1..18: note = antiviral peptide candidate (or antiviral peptide)
LSVAGWLDTIWDAIKRFF

SEQ ID NO: 210 - protein, 18 aa, synthetic construct
  source 1..18: note = antiviral peptide candidate (or antiviral peptide)
FAKDIWRILVAWTTTLWD

SEQ ID NO: 211 - protein, 18 aa, synthetic construct
  source 1..18: note = antiviral peptide candidate (or antiviral peptide)
KDIITVIAKYFGFIIEFL

SEQ ID NO: 212 - protein, 18 aa, synthetic construct
  source 1..18: note = antiviral peptide candidate (or antiviral peptide)
FEFLSRMVDSLVSFLSEF

SEQ ID NO: 213 - protein, 18 aa, synthetic construct
  source 1..18: note = antiviral peptide candidate (or antiviral peptide)
FEIIHGLLDRIMQLLDVL

SEQ ID NO: 214 - protein, 18 aa, synthetic construct
  source 1..18: note = antiviral peptide candidate (or antiviral peptide)
MLGLMDELIQMIDALVRI

SEQ ID NO: 215 - protein, 18 aa, synthetic construct
  source 1..18: note = antiviral peptide candidate (or antiviral peptide)
FFDFFVEDFSRWYIQIIR

SEQ ID NO: 216 - protein, 18 aa, synthetic construct
  source 1..18: note = antiviral peptide candidate (or antiviral peptide)
QLLLRALDAVATCWEKLF

SEQ ID NO: 217 - protein, 18 aa, synthetic construct
  source 1..18: note = antiviral peptide candidate (or antiviral peptide)
ILEWFTNYIRSWEEVFKL

SEQ ID NO: 218 - protein, 18 aa, synthetic construct
  source 1..18: note = antiviral peptide candidate (or antiviral peptide)
ILVSQWVEYLKIFENFFK

SEQ ID NO: 219 - protein, 18 aa, synthetic construct
  source 1..18: note = antiviral peptide candidate (or antiviral peptide)
FFEKIMSHIKNLLEWLGV

SEQ ID NO: 220 - protein, 18 aa, synthetic construct
  source 1..18: note = antiviral peptide candidate (or antiviral peptide)
LQMLGDFERAWSLILEFI

SEQ ID NO: 221 - protein, 18 aa, synthetic construct
  source 1..18: note = antiviral peptide candidate (or antiviral peptide)
ILVRWLSHFFEYLDRFYT

SEQ ID NO: 222 - protein, 18 aa, synthetic construct
  source 1..18: note = antiviral peptide candidate (or antiviral peptide)
FGDLLGEFWLGLKKIFYI

SEQ ID NO: 223 - protein, 18 aa, synthetic construct
  source 1..18: note = antiviral peptide candidate (or antiviral peptide)
MYAVIGFLDDFLKVFKQI

SEQ ID NO: 224 - protein, 18 aa, synthetic construct
  source 1..18: note = antiviral peptide candidate (or antiviral peptide)
VWDEFLVLLSKLMEIVNN

SEQ ID NO: 225 - protein, 18 aa, synthetic construct
  source 1..18: note = antiviral peptide candidate (or antiviral peptide)
MEKILEIIRVILKLYEQW

SEQ ID NO: 226 - protein, 18 aa, synthetic construct
  source 1..18: note = antiviral peptide candidate (or antiviral peptide)
DKIFTDIFHYLEVLFRII

SEQ ID NO: 227 - protein, 18 aa, synthetic construct
  source 1..18: note = antiviral peptide candidate (or antiviral peptide)
FLDNIDFLFMFIVKFLDK

SEQ ID NO: 228 - protein, 18 aa, synthetic construct
  source 1..18: note = antiviral peptide candidate (or antiviral peptide)
FLEDVVIYISRLLRLWIS

SEQ ID NO: 229 - protein, 18 aa, synthetic construct
  source 1..18: note = antiviral peptide candidate (or antiviral peptide)
INDLFSEILMSFLKFLDL

SEQ ID NO: 230 - protein, 18 aa, synthetic construct
  source 1..18: note = antiviral peptide candidate (or antiviral peptide)
LKTFISTVNELFEWVIRL

SEQ ID NO: 231 - protein, 18 aa, synthetic construct
  source 1..18: note = antiviral peptide candidate (or antiviral peptide)
WLSGIYEFFLRYKNIWVE

SEQ ID NO: 232 - protein, 18 aa, synthetic construct
  source 1..18: note = antiviral peptide candidate (or antiviral peptide)
LKIYYEIMDFIDFVLSKW

SEQ ID NO: 233 - protein, 18 aa, synthetic construct
  source 1..18: note = antiviral peptide candidate (or antiviral peptide)
FTYIDDLVEGIVKLIGVI

SEQ ID NO: 234 - protein, 18 aa, synthetic construct
  source 1..18: note = antiviral peptide candidate (or antiviral peptide)
VLVYFWRDYIEIIVKGIT

SEQ ID NO: 235 - protein, 18 aa, synthetic construct
  source 1..18: note = antiviral peptide candidate (or antiviral peptide)
FVDIVFGLLEGWWRFADG

SEQ ID NO: 236 - protein, 18 aa, synthetic construct
  source 1..18: note = antiviral peptide candidate (or antiviral peptide)
QLSILFTDWLEWFDKILA

SEQ ID NO: 237 - protein, 18 aa, synthetic construct
  source 1..18: note = antiviral peptide candidate (or antiviral peptide)
FWMGVIGFLDDYMKVVLK

SEQ ID NO: 238 - protein, 18 aa, synthetic construct
  source 1..18: note = antiviral peptide candidate (or antiviral peptide)
GEMASQFVTFLEKWFELF

SEQ ID NO: 239 - protein, 18 aa, synthetic construct
  source 1..18: note = antiviral peptide candidate (or antiviral peptide)
GFFFGWIGLLEGIIREIK

SEQ ID NO: 240 - protein, 18 aa, synthetic construct
  source 1..18: note = antiviral peptide candidate (or antiviral peptide)
FFSMVRDLLSWMESIIRQ

SEQ ID NO: 241 - protein, 18 aa, synthetic construct
  source 1..18: note = antiviral peptide candidate (or antiviral peptide)
GIHALWRIFDDWADIFVV

SEQ ID NO: 242 - protein, 18 aa, synthetic construct
  source 1..18: note = antiviral peptide candidate (or antiviral peptide)
GRWIDMLISRIFDIMLAF

SEQ ID NO: 243 - protein, 18 aa, synthetic construct
  source 1..18: note = antiviral peptide candidate (or antiviral peptide)
HEVMEFIEKLFLYIFKTI

SEQ ID NO: 244 - protein, 18 aa, synthetic construct
  source 1..18: note = antiviral peptide candidate (or antiviral peptide)
HLLKDWTDTFVYILEKLI

SEQ ID NO: 245 - protein, 18 aa, synthetic construct
  source 1..18: note = antiviral peptide candidate (or antiviral peptide)
HTLLDFWRLVWEFGVKVI

SEQ ID NO: 246 - protein, 18 aa, synthetic construct
  source 1..18: note = antiviral peptide candidate (or antiviral peptide)
HWSKLLEEIQALIKLLLA

SEQ ID NO: 247 - protein, 18 aa, synthetic construct
  source 1..18: note = antiviral peptide candidate (or antiviral peptide)
IDDILTILLRLQKGLLGL

SEQ ID NO: 248 - protein, 18 aa, synthetic construct
  source 1..18: note = antiviral peptide candidate (or antiviral peptide)
IEHLEQLFWRIFRNIVLF

SEQ ID NO: 249 - protein, 18 aa, synthetic construct
  source 1..18: note = antiviral peptide candidate (or antiviral peptide)
IQVFADVFKMLIKEIITI

SEQ ID NO: 250 - protein, 18 aa, synthetic construct
  source 1..18: note = antiviral peptide candidate (or antiviral peptide)
VAFGIIGFIDDFIKVILK

SEQ ID NO: 251 - protein, 18 aa, synthetic construct
  source 1..18: note = antiviral peptide candidate (or antiviral peptide)
IIGWIDHFQNWLEKLHKL

SEQ ID NO: 252 - protein, 18 aa, synthetic construct
  source 1..18: note = antiviral peptide candidate (or antiviral peptide)
VLYKEVLKTIIDLIENII

SEQ ID NO: 253 - protein, 18 aa, synthetic construct
  source 1..18: note = antiviral peptide candidate (or antiviral peptide)
IIISLLKQLLKTYGDLID

SEQ ID NO: 254 - protein, 18 aa, synthetic construct
  source 1..18: note = antiviral peptide candidate (or antiviral peptide)
IIYQVIDELVNYFKKFLF

SEQ ID NO: 255 - protein, 18 aa, synthetic construct
  source 1..18: note = antiviral peptide candidate (or antiviral peptide)
IKIINQWEALLKEFTSLI

SEQ ID NO: 256 - protein, 18 aa, synthetic construct
  source 1..18: note = antiviral peptide candidate (or antiviral peptide)
VTIYEMVLKSLLEIFKIL

SEQ ID NO: 257 - protein, 18 aa, synthetic construct
  source 1..18: note = antiviral peptide candidate (or antiviral peptide)
ILKDLLHWFKTQFFTWFD

SEQ ID NO: 258 - protein, 18 aa, synthetic construct
  source 1..18: note = antiviral peptide candidate (or antiviral peptide)
TIWLGFIGFMDDYIKVFK

SEQ ID NO: 259 - protein, 18 aa, synthetic construct
  source 1..18: note = antiviral peptide candidate (or antiviral peptide)
INALFDVWIDVQRRWVYL

SEQ ID NO: 260 - protein, 18 aa, synthetic construct
  source 1..18: note = antiviral peptide candidate (or antiviral peptide)
IWRRWLYVLWDEVAQLVN

SEQ ID NO: 261 - protein, 18 aa, synthetic construct
  source 1..18: note = antiviral peptide candidate (or antiviral peptide)
LNDIVIIMKSIIYEWFDI

SEQ ID NO: 262 - protein, 18 aa, synthetic construct
  source 1..18: note = antiviral peptide candidate (or antiviral peptide)
IRVMFDEITRILNHLLGI

SEQ ID NO: 263 - protein, 18 aa, synthetic construct
  source 1..18: note = antiviral peptide candidate (or antiviral peptide)
TTWWNILERIDHKLFMWI

SEQ ID NO: 264 - protein, 18 aa, synthetic construct
  source 1..18: note = antiviral peptide candidate (or antiviral peptide)
LSEWLRIIEFLLQGLKVY

SEQ ID NO: 265 - protein, 18 aa, synthetic construct
  source 1..18: note = antiviral peptide candidate (or antiviral peptide)
WLLLFSEWLGNLQKIFDE

SEQ ID NO: 266 - protein, 18 aa, synthetic construct
  source 1..18: note = antiviral peptide candidate (or antiviral peptide)
RVILGAIERFIGVLIEHF

SEQ ID NO: 267 - protein, 18 aa, synthetic construct
  source 1..18: note = antiviral peptide candidate (or antiviral peptide)
KILDQWFFRITAYIDELL

SEQ ID NO: 268 - protein, 18 aa, synthetic construct
  source 1..18: note = antiviral peptide candidate (or antiviral peptide)
IYIFFRHWTTIYERLLEI

SEQ ID NO: 269 - protein, 18 aa, synthetic construct
  source 1..18: note = antiviral peptide candidate (or antiviral peptide)
VFWYFWEDLTGIAKGIIK

SEQ ID NO: 270 - protein, 18 aa, synthetic construct
  source 1..18: note = antiviral peptide candidate (or antiviral peptide)
KEFFTELFILLKSIFSFV

SEQ ID NO: 271 - protein, 18 aa, synthetic construct
  source 1..18: note = antiviral peptide candidate (or antiviral peptide)
KELWLNIVNIILTLYEDL

SEQ ID NO: 272 - protein, 18 aa, synthetic construct
  source 1..18: note = antiviral peptide candidate (or antiviral peptide)
KILNQITLFWMDMFKDII

SEQ ID NO: 273 - protein, 18 aa, synthetic construct
  source 1..18: note = antiviral peptide candidate (or antiviral peptide)
KLFSKLIDILDDYYVLLV

SEQ ID NO: 274 - protein, 18 aa, synthetic construct
  source 1..18: note = antiviral peptide candidate (or antiviral peptide)
LDKVMKIWTTFVEQIFGV

SEQ ID NO: 275 - protein, 18 aa, synthetic construct
  source 1..18: note = antiviral peptide candidate (or antiviral peptide)
LDVLSSIGQLIRDILDFI

SEQ ID NO: 276 - protein, 18 aa, synthetic construct
  source 1..18: note = antiviral peptide candidate (or antiviral peptide)
LEKIYDIIGYIYQYLKLL

SEQ ID NO: 277 - protein, 18 aa, synthetic construct
  source 1..18: note = antiviral peptide candidate (or antiviral peptide)
LVFFSKVLQYLIEELLEI

SEQ ID NO: 278 - protein, 18 aa, synthetic construct
  source 1..18: note = antiviral peptide candidate (or antiviral peptide)
LISFIDYISEIIANIIDR

SEQ ID NO: 279 - protein, 18 aa, synthetic construct
  source 1..18: note = antiviral peptide candidate (or antiviral peptide)
LITMVLTMIQWWRDVIRE

SEQ ID NO: 280 - protein, 18 aa, synthetic construct
  source 1..18: note = antiviral peptide candidate (or antiviral peptide)
LVMIVATMIQWWRDVIRE

SEQ ID NO: 281 - protein, 18 aa, synthetic construct
  source 1..18: note = antiviral peptide candidate (or antiviral peptide)
SLLTLILEQFDDLLVKIL

SEQ ID NO: 282 - protein, 18 aa, synthetic construct
  source 1..18: note = antiviral peptide candidate (or antiviral peptide)
LLKEILNLYLDLGTWLLK

SEQ ID NO: 283 - protein, 18 aa, synthetic construct
  source 1..18: note = antiviral peptide candidate (or antiviral peptide)
WEKLMLLIIDLFKFLDQY

SEQ ID NO: 284 - protein, 18 aa, synthetic construct
  source 1..18: note = antiviral peptide candidate (or antiviral peptide)
LQELMKVLIDWINDVLVG

SEQ ID NO: 285 - protein, 18 aa, synthetic construct
  source 1..18: note = antiviral peptide candidate (or antiviral peptide)
LWLSWEEGLQHFLKYLLD

SEQ ID NO: 286 - protein, 18 aa, synthetic construct
  source 1..18: note = antiviral peptide candidate (or antiviral peptide)
LWNDIMQFVEQFFWRLVE

SEQ ID NO: 287 - protein, 18 aa, synthetic construct
  source 1..18: note = antiviral peptide candidate (or antiviral peptide)
LYEFFQAYKTVWTEIWKI

SEQ ID NO: 288 - protein, 18 aa, synthetic construct
  source 1..18: note = antiviral peptide candidate (or antiviral peptide)
MLIERLIDAINSWVQLIE

SEQ ID NO: 289 - protein, 18 aa, synthetic construct
  source 1..18: note = antiviral peptide candidate (or antiviral peptide)
QIWNMVIELLDQVVEVFK

SEQ ID NO: 290 - protein, 18 aa, synthetic construct
  source 1..18: note = antiviral peptide candidate (or antiviral peptide)
YVVTFVELVWNIIEKLLD

SEQ ID NO: 291 - protein, 18 aa, synthetic construct
  source 1..18: note = antiviral peptide candidate (or antiviral peptide)
REVHEIWASLIEIALSLW

SEQ ID NO: 292 - protein, 18 aa, synthetic construct
  source 1..18: note = antiviral peptide candidate (or antiviral peptide)
RVIHQFLELWYRYVVEVL

SEQ ID NO: 293 - protein, 18 aa, synthetic construct
  source 1..18: note = antiviral peptide candidate (or antiviral peptide)
TDIIDIIDQIVILLTKFI

SEQ ID NO: 294 - protein, 18 aa, synthetic construct
  source 1..18: note = antiviral peptide candidate (or antiviral peptide)
TLTDWKTWISFWKTLIDW

SEQ ID NO: 295 - protein, 18 aa, synthetic construct
  source 1..18: note = antiviral peptide candidate (or antiviral peptide)
WFEAVLGYISAVVELFRE

SEQ ID NO: 296 - protein, 18 aa, synthetic construct
  source 1..18: note = antiviral peptide candidate (or antiviral peptide)
WIESILELIKKHLLSLWN

SEQ ID NO: 297 - protein, 18 aa, synthetic construct
  source 1..18: note = antiviral peptide candidate (or antiviral peptide)
WLAWIDWIRGLDGQLIKI

SEQ ID NO: 298 - protein, 18 aa, synthetic construct
  source 1..18: note = antiviral peptide candidate (or antiviral peptide)
YEIIKWTSFLLEYLTEII

SEQ ID NO: 299 - protein, 18 aa, synthetic construct
  source 1..18: note = antiviral peptide candidate (or antiviral peptide)
YGELNIFWLQILEIIRRW

SEQ ID NO: 300 - protein, 18 aa, synthetic construct
  source 1..18: note = antiviral peptide candidate (or antiviral peptide)
FKLIWGSIFSFLEQIEKF

SEQ ID NO: 301 - protein, 18 aa, synthetic construct
  source 1..18: note = antiviral peptide
DWLRIIWDWVCSVVSDFK

SEQ ID NO: 302 - DNA, 24 bp, synthetic construct
  source 1..24: mol_type = other DNA; note = forward primer
gaaagaccagagatcctgctgtct

SEQ ID NO: 303 - DNA, 21 bp, synthetic construct
  source 1..21: mol_type = other DNA; note = reverse primer
accattccattttctggcgtt

SEQ ID NO: 304 - DNA, 17 bp, synthetic construct
  source 1..17: mol_type = other DNA; note = probe
agcatcattccaggcac